European Patent Specification EP 3 332 633 B1, published June 28, 2023. Title: Plants Having mutated cyclin F-box gene. Applicant: University of Tsukuba. The sequence listing filed with the application follows.

SEQUENCE LISTING (22 sequences)

SEQ ID NO: 1 - DNA, 1215 bp, Solanum lycopersicum
  CDS (1)..(1215)
  CDS sequence encoding wild-type cyclin F-box protein
atggaagaaacctcttgggtcagtcattgccctgattacgttgtaccagacatggttgagtttgattcattttcagagcttaatgatgaagaaaatagagaggcttcctcagttcctgtggatttgatactgcctgatgatttactggaacgcatactggcctatcttcccattgccagcatttttagggcaagttgtgtgtgtaaaagatggtgtgagatagtgaattcaagaaggtttttatggaacttctctcaggtgctgtctcaaaaaccgtggtactttatgttcacaagctcagaggagccagttggttatgcctatgatccttcccttcgaaaatggtatagtattgacctcccttgcattcagacatcaaattggttcattgcttcttcatgtggattagtttgcatcatggacaatgacagtagaagcgaactatatgtttgtaacccaataaccaaatgcagcaagaaccttcaggagcctcctggtctcaagttttctgattacagtgcattggctatctgtgcaaacatgaaaacttcttgttacagtgtcgccattgttaaatctaagcaagtacctggtaacttctatcagtgggatctctcaatccacatatatgattctggaacaatgaagtggttgacccctttgacagaggttctaacaggctggagaggtggggatgaaagtgtcatctgtgatggtgttttgtacttcctgatctatgcaactggaggtggtggtctagaaagtcgtcatggtctgatcacttacaacctctcaagcagatcatcccattgttcgttaataaagactttcattcccgtgccatgttctctaacatgtggtcgattgatgaacctcaaggagaagttagtaatggtgggagggattgggaaaccagaccgtcctgacataattaaggggattggcatatgggcacttcaggggacagaatggcaagaaattgcccgcatgccacacaagtattttcaaggttttggggaattcgatgatgtttttgccagcagtggcactgatgatctcatatacattcagagttatggagctcctgcccttcttgtttttgacgtgaaccagaaacagtggaggtggtcacagaaatgtccagtgacaaagaggtttccccttcagctctttactggtttctgcttcgagccaaggcttgagatgtctccctga

SEQ ID NO: 2 - protein, 404 aa, Solanum lycopersicum
  Amino acid sequence of wild-type cyclin F-box protein
MEETSWVSHCPDYVVPDMVEFDSFSELNDEENREASSVPVDLILPDDLLERILAYLPIASIFRASCVCKRWCEIVNSRRFLWNFSQVLSQKPWYFMFTSSEEPVGYAYDPSLRKWYSIDLPCIQTSNWFIASSCGLVCIMDNDSRSELYVCNPITKCSKNLQEPPGLKFSDYSALAICANMKTSCYSVAIVKSKQVPGNFYQWDLSIHIYDSGTMKWLTPLTEVLTGWRGGDESVICDGVLYFLIYATGGGGLESRHGLITYNLSSRSSHCSLIKTFIPVPCSLTCGRLMNLKEKLVMVGGIGKPDRPDIIKGIGIWALQGTEWQEIARMPHKYFQGFGEFDDVFASSGTDDLIYIQSYGAPALLVFDVNQKQWRWSQKCPVTKRFPLQLFTGFCFEPRLEMSP

SEQ ID NO: 3 - DNA, 1215 bp, Solanum lycopersicum
  CDS (1)..(1215)
  CDS sequence encoding mutant cyclin F-box protein (from E8986)
atggaagaaacctcttgggtcagtcattgccctgattacgttgtaccagacatggttgagtttgattcattttcagagcttaatgatgaagaaaatagagaggcttcctcagttcctgtggatttgatactgcctgatgatttactggaacgcatactggcctatcttcccattgccagcatttttagggcaagttgtgtgtgtaaaagatggtgtgagatagtgaattcaagaaggtttttatggaacttctctcaggtgctgtctcaaaaaccgtggtactttatgttcacaagctcagaggagccagttggttatgcctatgatccttcccttcgaaaatggtatagtattgacctcccttgcattcagacatcaaattggttcattgcttcttcatgtggattagtttgcatcatggacaatgacagtagaagcgaactatatgtttgtaacccaataaccaaatgcagcaagaaccttcaggagcctcctggtctcaagttttctgattacagtgcattggctatctgtgcaaacatgaaaacttcttgttacagtgtcgccattgttaaatctaagcaagtacctggtaacttctatcagtgggatctctcaatccacatatatgattctggaacaatgaagtggttgacccctttgacagaggttctaacaggctggagaggtggggatgaaagtgtcatctgtgatggtgttttgtacttcctgatctatgcaactggaggtggtggtctagaaagtcgtcatggtctgatcacttacaacctctcaagcagatcatcccattgttcgttaataaagactttcattcccgtgccatgttctctaacatgtggtcgattgatgaacctcaaggagaagttagtaatggtgggagggattgggaaaccagaccgtcctgacataattaaggggattggcatatgggcacttcaggggacagaatggcaagaaattgcccgcatgccacacaagtattttcaaggttttggggaattcgatgatgtttttgccagcagtggcactgatgatctcatatacattcagagttatggagctcctgcccttcttgtttttgacgtgaaccagaaacagtggaggtggtcacagaaatgtccagtgacaaagaggtttccccttcagctctttactggtttctgcttcgagcaaaggcttgagatgtctccctga

SEQ ID NO: 4 - protein, 404 aa, Solanum lycopersicum
  Amino acid sequence of mutant cyclin F-box protein (from E8986)
MEETSWVSHCPDYVVPDMVEFDSFSELNDEENREASSVPVDLILPDDLLERILAYLPIASIFRASCVCKRWCEIVNSRRFLWNFSQVLSQKPWYFMFTSSEEPVGYAYDPSLRKWYSIDLPCIQTSNWFIASSCGLVCIMDNDSRSELYVCNPITKCSKNLQEPPGLKFSDYSALAICANMKTSCYSVAIVKSKQVPGNFYQWDLSIHIYDSGTMKWLTPLTEVLTGWRGGDESVICDGVLYFLIYATGGGGLESRHGLITYNLSSRSSHCSLIKTFIPVPCSLTCGRLMNLKEKLVMVGGIGKPDRPDIIKGIGIWALQGTEWQEIARMPHKYFQGFGEFDDVFASSGTDDLIYIQSYGAPALLVFDVNQKQWRWSQKCPVTKRFPLQLFTGFCFEQRLEMSP

SEQ ID NO: 5 - DNA, 22 bp, Artificial
  primer
cccgcatgccacacaagtattt

SEQ ID NO: 6 - DNA, 30 bp, Artificial
  primer
atcacatatcagggagacatctcaagccat

SEQ ID NO: 7 - DNA, 20 bp, Artificial
  primer
ggaaaccagaccgtcctgac

SEQ ID NO: 8 - DNA, 20 bp, Artificial
  primer
tgcattgagaggagctaggg

SEQ ID NO: 9 - DNA, 267 bp, Solanum lycopersicum
  analyzed sequence of wild-type Micro-Tom
tgggcacttcaggggacagaatggcaagaaattgcccgcatgccacacaagtattttcaaggttttggggaattcgatgatgtttttgccagcagtggcactgatgatctcatatacattcagagttatggagctcctgcccttcttgtttttgacgtgaaccagaaacagtggaggtggtcacagaaatgtccagtgacaaagaggtttccccttcagctctttactggtttctgcttcgagccaaggcttgagatgtctccctga

SEQ ID NO: 10 - DNA, 267 bp, Solanum lycopersicum
  analyzed sequence of mutant Micro-Tom (E8986)
tgggcacttcaggggacagaatggcaagaaattgcccgcatgccacacaagtattttcaaggttttggggaattcgatgatgtttttgccagcagtggcactgatgatctcatatacattcagagttatggagctcctgcccttcttgtttttgacgtgaaccagaaacagtggaggtggtcacagaaatgtccagtgacaaagaggtttccccttcagctctttactggtttctgcttcgagcaaaggcttgagatgtctccctga

SEQ ID NO: 11 - DNA, 20 bp, Artificial
  primer
ccacagccttagggttggag

SEQ ID NO: 12 - DNA, 20 bp, Artificial
  primer
acggtctggtttcccaatcc

SEQ ID NO: 13 - DNA, 22 bp, Artificial
  primer
gcattggctatctgtgcaaaca

SEQ ID NO: 14 - DNA, 22 bp, Artificial
  primer
agacaacttgtccctgtcttgg

SEQ ID NO: 15 - DNA, 22 bp, Artificial
  primer
ttctggaacaatgaagtggttg

SEQ ID NO: 16 - DNA, 36 bp, Artificial
  primer
ccttaattatgtcaggacggtctggtttcacaatcc

SEQ ID NO: 17 - DNA, 44 bp, Artificial
  primer
ttcattttcagagcttaatgatgaagaaaatagagaggcttccc

SEQ ID NO: 18 - DNA, 23 bp, Artificial
  primer
tgaatgcaagggaggtcaatact

SEQ ID NO: 19 - DNA, 1215 bp, Solanum lycopersicum
  CDS (1)..(1215)
  CDS sequence encoding wild-type cyclin F-box protein (from W3583)
atggaagaaacctcttgggtcagtcattgccctgattacgttgtaccagacatggttgagtttgattcattttcagagcttaatgatgaagaaaatagagaggcttccttagttcctgtggatttgatactgcctgatgatttactggaacgcatactggcctatcttcccattgccagcatttttagggcaagttgtgtgtgtaaaagatggtgtgagatagtgaattcaagaaggtttttatggaacttctctcaggtgctgtctcaaaaaccgtggtactttatgttcacaagctcagaggagccagttggttatgcctatgatccttcccttcgaaaatggtatagtattgacctcccttgcattcagacatcaaattggttcattgcttcttcatgtggattagtttgcatcatggacaatgacagtagaagcgaactatatgtttgtaacccaataaccaaatgcagcaagaaccttcaggagcctcctggtctcaagttttctgattacagtgcattggctatctgtgcaaacatgaaaacttcttgttacagtgtcgccattgttaaatctaagcaagtacctggtaacttctatcagtgggatctctcaatccacatatatgattctggaacaatgaagtggttgacccctttgacagaggttctaacaggctggagaggtggggatgaaagtgtcatctgtgatggtgttttgtacttcctgatctatgcaactggaggtggtggtctagaaagtcgtcatggtctgatcacttacaacctctcaagcagatcatcccattgttcgttaataaagactttcattcccgtgccatgttctctaacatgtggtcgattgatgaacctcaaggagaagttagtaatggtgggagggattgggaaaccagaccgtcctgacataattaaggggattggcatatgggcacttcaggggacagaatggcaagaaattgcccgcatgccacacaagtattttcaaggttttggggaattcgatgatgtttttgccagcagtggcactgatgatctcatatacattcagagttatggagctcctgcccttcttgtttttgacgtgaaccagaaacagtggaggtggtcacagaaatgtccagtgacaaagaggtttccccttcagctctttactggtttctgcttcgagccaaggcttgagatgtctccctga

SEQ ID NO: 20 - protein, 404 aa, Solanum lycopersicum
  Amino acid sequence of wild-type cyclin F-box protein
MEETSWVSHCPDYVVPDMVEFDSFSELNDEENREASLVPVDLILPDDLLERILAYLPIASIFRASCVCKRWCEIVNSRRFLWNFSQVLSQKPWYFMFTSSEEPVGYAYDPSLRKWYSIDLPCIQTSNWFIASSCGLVCIMDNDSRSELYVCNPITKCSKNLQEPPGLKFSDYSALAICANMKTSCYSVAIVKSKQVPGNFYQWDLSIHIYDSGTMKWLTPLTEVLTGWRGGDESVICDGVLYFLIYATGGGGLESRHGLITYNLSSRSSHCSLIKTFIPVPCSLTCGRLMNLKEKLVMVGGIGKPDRPDIIKGIGIWALQGTEWQEIARMPHKYFQGFGEFDDVFASSGTDDLIYIQSYGAPALLVFDVNQKQWRWSQKCPVTKRFPLQLFTGFCFEPRLEMSP

SEQ ID NO: 21 - DNA, 1215 bp, Solanum lycopersicum
  CDS (1)..(1215)
  CDS sequence encoding wild-type cyclin F-box protein (from W283)
atggaagaaacctcttgggtcagtcattgccctgattacgttgtaccagacatggttgagtttgattcattttcagagcttaatgatgaagaaaatagagaggcttcctcagttcctgtggatttgatactgcctgatgatttactggaacgcatactggcctatcttcccattgccagcatttttagggcaagttgtgtgtgtaaaagatggtgtgagatagtgaattcaagaaggtttttatggaacttctctcaggtgctgtctcaaaaaccgtggtactttatgttcacaagctcagaggagccagttggttatgcctatgatccttcccttcgaaaatggtatagtattgacctcccttgcattcagacatcaaattggttcattgcttcttcatgtggattagtttgcatcatggacaatgacagtagaagcgaactatatgtttgtaacccaataaccaaatgcagcaagaaccttcaggagcctcctggtctcaagttttctgattacagtgcattggctatctgtgcaaacatgaaaacttcttgttacagtgtcgccattgttaaatctaagcaagtacctggtaacttctatcagtgggatctctcaatccacatatatgattctggaacaatgaagtggttgacccctttgacagaggttctaacaggctggagaggtggggatgaaagtgtcatctgtgatggtgttttgtacttcctgatctatgcaactggaggtggtggtctagaaagtcgtcatggtctgatcacttacaacctctcaagcagatcatcccattgttcgttaataaagactttcattcccgtgccatgttctctaacatgtggtcgattgatgaacctcaaggagaagttagtaatggtgggaaggattgggaaaccagaccgtcctgacataattaaggggattggcatatgggcacttcaggggacagaatggcaagaaattgcccgcatgccacacaagtattttcaaggttttggggaattcgatgatgtttttgccagcagtggcactgatgatctcatatacattcagagttatggagctcctgcccttcttgtttttgacgtgaaccagaaacagtggaggtggtcacagaaatgtccagtgacaaagaggtttccccttcagctctttactggtttctgcttcgagccaaggcttgagatgtctccctga

SEQ ID NO: 22 - protein, 404 aa, Solanum lycopersicum
  Amino acid sequence of wild-type cyclin F-box protein (from W283)
MEETSWVSHCPDYVVPDMVEFDSFSELNDEENREASSVPVDLILPDDLLERILAYLPIASIFRASCVCKRWCEIVNSRRFLWNFSQVLSQKPWYFMFTSSEEPVGYAYDPSLRKWYSIDLPCIQTSNWFIASSCGLVCIMDNDSRSELYVCNPITKCSKNLQEPPGLKFSDYSALAICANMKTSCYSVAIVKSKQVPGNFYQWDLSIHIYDSGTMKWLTPLTEVLTGWRGGDESVICDGVLYFLIYATGGGGLESRHGLITYNLSSRSSHCSLIKTFIPVPCSLTCGRLMNLKEKLVMVGRIGKPDRPDIIKGIGIWALQGTEWQEIARMPHKYFQGFGEFDDVFASSGTDDLIYIQSYGAPALLVFDVNQKQWRWSQKCPVTKRFPLQLFTGFCFEPRLEMSP